European Patent Specification EP 4 010 473 B1, published November 20, 2024. Title: COMPOSITIONS AND METHODS FOR DETECTING METHYLATED DNA. Applicant: Spurbeck, Rachel. The sequence listing filed with the application follows.

SEQUENCE LISTING (9 sequences)

SEQ ID NO: 1 - DNA, 12 bp, Artificial Sequence
  Restriction site target sequence
  misc_feature (6)..(9): n is a, c, g, or t
cgatcnnnntgc

SEQ ID NO: 2 - DNA, 10 bp, Artificial Sequence
  Restriction site target sequence
  misc_feature (4)..(5): n is a, c, g, or t
cagnncctgg

SEQ ID NO: 3 - DNA, 10 bp, Artificial Sequence
  Restriction site target sequence
  misc_feature (5)..(7): n is a, c, g, or t
gatcnnnatc

SEQ ID NO: 4 - DNA, 11 bp, Artificial Sequence
  Restriction site target sequence
  misc_feature (6)..(9): n is a, c, g, or t
ccwggnnnngg

SEQ ID NO: 5 - DNA, 12 bp, Artificial Sequence
  Restriction site target sequence
  misc_feature (6)..(9): n is a, c, g, or t
ccaggnnnntgg

SEQ ID NO: 6 - DNA, 11 bp, Artificial Sequence
  Restriction site target sequence
ggccggccwgg

SEQ ID NO: 7 - DNA, 11 bp, Artificial Sequence
  Restriction site target sequence
  misc_feature (6)..(8): n is a, c, g, or t
ccaggnnntgg

SEQ ID NO: 8 - DNA, 13 bp, Artificial Sequence
  Restriction site target sequence
  misc_feature (8)..(9): n is a, c, g, or t
ggccwggnnggcc

SEQ ID NO: 9 - DNA, 16 bp, Artificial Sequence
  Restriction site target sequence
  misc_feature (5)..(9): n is a, c, g, or t
ggccnnnnnggccwgg